European Patent Specification EP 3 442 551 B1, published February 7, 2024. Title: A BACTERIOPHAGE STRAIN CAPABLE OF PRODUCING A LYTIC INFECTION IN THE ESCHERICHIA COLI ST131-O25B:H4 CLONE. Applicant: Inserm. The sequence listing filed with the application follows.

SEQUENCE LISTING (2 sequences)

SEQ ID NO: 1 - protein, 726 aa, Artificial Sequence
  bacteriophage tail fiber
MSTITQFPSGNTQYRIEFDYLARTFVVVTLVNSSNPTLNRVLEVGRDYRFLNPTMIEMLADQSGFDIVRIHRQTGTDLVVDFRNGSVLTASDLTNSELQAIHIAEEGRDQTVDLAKEYADAAGSSAGNAKDSEDESRRIAASIKAAGKIGYITRRSFEKGFNVTTWNEVLLWEEDGDYYRWDGTLPKNVPAGSTPESSGGIGLSAWVSVGDASLRANLADSDGAKYIGSGERTLLEHNNDVLHSKDFPTLQAAIDASLQKNDLLVSPGNYTEKVTIGNAQLKGVGGATVLKTPADFTNTVQVNLATPHWQFRHSGGFAIDGSGTTGAVGISFDPSDQYSGRHNFSDVYIHNINKAIQKPSGNIGNTWRNIGISTCDWGYYAISGSEMHCGADTLYNIHFDGISTYAVYLDGTVDNGGGGAWWLKDSIIEASGGGGIYLKSKSGDCPTSPCGVSNIWMEAIATSPAVQVDGVAQKPRVLKLVDTAIFFAEYSYLNNIELSNSNLVTYGCRFDNADGNQDIVVDAQSTIVAHDVYLNGSSGKDVIVESVASQSATIAATNLSLRGNLTRGRVFNTPTGNKLMAITFDSGSHNFSGSGTVNGSTVSDGLHAATCTEFSFPGAGLYEMVATRTTITSGRWYVWGVNSRLQSGSADISITSGITMGSVYTKPGEWISTFGVGKASTTGTVALYVSTGGGSGATVRFSDFFIAEFTTQAQALAFANSRMSLS

SEQ ID NO: 2 - DNA, 38979 bp, Artificial Sequence
  the genomic sequence of LM33-P1
ttcaagaacctcaagtctccccataggccctctttcagtccagaccaaaggccctacccgttactgctccttgcagtcacagccagtctatcataaggttggacagatggtcaagacttaaggtcaacgataggctgaggctatggcttagggaaggacgataggttgggactattggtcttctttgagtctctatctgtataaccataagtcacaaccataggtcacagcctacctctcacaaccataagtcataacctacagtctcactaacctacagtctcaaccataagacaccaacacctacagtcatagacctacagttaatagacacaaggctatagacttaaggtctaagacatgttagtcaaagactatatcctcttacaccatggggccgacgatagcttaatcaatattatttcaaattacctattgactataggtccagactatggcctaatagcttccgtcaacacgacacggcaacaaccggatagtgaagacgccggtccggtccggttaagtagtcagcctgtaagacatacgaacaacaggcaaccgacagaaagtagttgacaggcagtaacgacttaaagtaatatgtaccacatcgaaacaacggtgatgaccaacactgaatggtctacctgaagtcctctgactgaagggaatgctctttaacaatctggataaactcttaatgtgcgccgatagcgactaactacagggcctttgagtctacatctgaaggccctgactgatagtcactaacttaaaggatggacactatgaaacacttaagcacaatcactaatcgcaatgaagtattcgtgaacactaaaggttatgcgtggattcagcttaaagagatgacaggagcgcgtcaccgtgtggtagtgcgcaaggtatcaagcaagcagttcagcaactacagcgtcgatactgtgcgtatagacaacgagacatacctgatagactcgcagataaccgtgagtcctacagtgggcgtctcagctccttatttcgctaactgagagtgattaactacaggtcgttagactgatagcggcctgactgatagtcactaacacataattaactttgagaggatataactatggaacgtaatgctaacgcatactatgagctgctggctgcaaccgttgaggcatttatcgagcgtattcagtacgaccacctgactcaagatgacgactacagcgctgcgctgcatgaggtcgtagacggtcaggttccacactattaccacgagatttttacggtgatggctgctgatggtatagacaacgagttcgaagactctgggatgatacctgaaaccaaggacgtaacgcgtatcctacaagctcgcatctatgaggcactttataacgacgtgtctaatagcttggatgtagtctggtttgaggatgaagaggcagacgaagaggatgaatattgggtagttgacgctaaaacaggcgcaataattgtgcaagctgtagctcttgaggtcgctactgcatgtgccaaggtcaactatgtgataggtcgccaccttcaggtggaagacatcaatgataacgtagtgtttgaccctgctgctgaggactgcgagtgatggtaacttatggcctctgccagcaccacgtcactaacgcccggcttatggtcaagaccgggcagttagaccacgattgggctatgcgtctcttgaaagtggtctacaggagacgcaagcgtatacacgacagtttacacgctaagtgacagactacaggtcatcaatgctggtggcctgactgatagtcattaacaactgagagggaagatatgaacacaatcactggtgccataaccaaaggttttcgagcaattttcggtgaaacgcaagaagtatgcaccaatcataaattcgtactttcttgcgtagcaggtgacgagtttgacgggttcgataaactggtggtttgcgaccattgcggacaagaggctatccaacactcaaacggtaaatttgaattaatagacgatagccttacagaaggagacggcgagtaacctaaataaacaggagagaaccaaatcatagcttgaccataacactgacgtgatggtactgagtgatagacgagaggtcatcgactgataggtggcctcaaagattaccacttacattgataggagttaactatgagcactgcaatcatctggactatctcaggcttcgtagcgtggggaatgtttactctagtctgcaaactaccggtccttactcaactgttatggggcttatgactatgagtatcgcactattgatagccataggctatggacttatcgcctacgtgctggtgagagacatcaacaaagcgcgtaaagtctacaaattcaaatatgtacgtctgggtagctggactgtacgtcaacctaacggacgattcatgcgtaacttagcgaacgtctgggatatagcaacacttgggagcaaactgtaatgaacaagtcatacgggattaatctggtacactctatggacgcagacatgcaaatgttaagcctactggctaccgggtatcgtcacggaacgtcaagtcactccgcacgtcaacagcaggagcgggaccgggtactgcaagcaagactccgggctgagggccataagtccgaactaatgtgtctggtgtatggtggacgaccaatcactgacgatggtaaacttttagtctcaggctggaaggcgatagaccaacggtcaaccatcaagcacacgactcatggtgacttcagtcatctccacgctaacccgctgatatgcaagtaattctgacttaactatcactataggactcaaggtctaagactccaagtgaaagaccaaagagactttaagtgaaagactaataacaaggactttaagtatgagcgtcatctctattgacaagcacgacttctctgatgtgtcgaacgccattgagccgtttaacctactggctgaccactacgggcaagacattgcagtcaaacagcttcagcttgagcacgaggcatacactgaaggcgagcgacgtttcatcaagaaccttgagagacagactgagcgaggggaactggcagacaatcaggtcgccaagcctttgatgcagactctggtccctaagattgcgcaagccgtcaaggagtggcatgaaggtccagacgggaagctgtcaacctctcgtccgagcgtagcgttcaccatgttgagcactgaagagaaggccgtaaaggtccgctctttgcgcatctcctgcgagtctgctgcggttatcatattgaaggtcatactctccaagctggtcaagcctgaagggataccgattacaccgatggcctcagcgataggtcgcacacttgaggacgaaatccgcttcggtcgcatccgtgacaaggagaaagagcacttcaagaaggcgatagctgataacctgaataagcgggccggggcgtcctacaagaaagcctacatgcaagcggtcgaggcatccatgctggagcaaggccaactggaagatgcgtgggggacttggagtccgaccgaggctgtccacgttggaatcaagatgctggagattgtcatccagtccacacaactggtcgagcttaagcgttacggtgctggcaatgcagcggctgacgttgagatggtccacctgtcagacttctgggtcaagaagatggcacaacgaggattcagccttgcgggtatagctccagtctaccagccttgcgtcgttccacctaagccgtggactggtgtcgtaggcggtgggtactgggccaaaggacgcagaccattaccactgattcgcttagggtctaagtctgcggtagcacgctacgaagacgtgtatatgcctgaagtctatgacgctgtgaacatcattcagaatacaccttggaaagtgaacaagaaggttctggaagtggtgaacatggtcgagaagctgaacaacacgcctattgatgacatccctcagatggaaccgctgaagcctgaggactatgcgggtgagactgaagaagaactcaaggcatggaagaaggctgctgctggtatctatcgccgcgagaaggccagacagtcacgaagattgtcactgagctttatcgtcaaccaagcgaacaagttctctcagttcaaggccatctggttcccgtataacatggactggcgcggtcgcgtctacgctgtgccgatgttcaaccctcagggtaacgacatgcaaaagggtcttctgactctggcagtcggtaagcctattggtgctgatggtttcaaatggctgaaggtccacggtgcaaactgcgcgggtgtcgataaagtcaccttcgaggagcgtatcaagtgggtggaagataaccacgacaacatcatggctgctgccaaggcaccgatggatagcattgagtggtggggcaagttagactctccgttctgcttcctagcgttctgcttcgagtatgctggcgtaatgcaccacggcttgtcttactcctgctcgctgccgatagcgttcgatgggtcctgctctgggattcagcacttcagcgctatgcttcgcgaccacatcggtggacatgcagtaaacctgacgccatccggtaaggtccaagacatctaccgcatcgtgtctgaccgcattgaggaggagcttaaagtcctactggttaacggtacggacaacgagatggtaactcacgaggacaagaaaactggtgagattaccgagcgtctcaagctggggacacgagagcttgcccgtcagtggctgacctacggtatgtcacgaaaggtcactaagcgttcggtcatgactctggcctacgggtcgaaagagtacggctgaggacatcgtgatgccagggacatcgtgatgccagcgattgactcagggtctggcgctatgttcactgaaccaagccaagcatctcgcttcatggctaagatgatttgggaagctgtgagtgtgaccgtagttgctgcggttgacgcgatgaaatggcttcagggtgctgccaagctgcttgctgctgaagtgaaggacaagaagactggagaaatcctgaagccttgtcttccggtacactgggtcacacctgatggtttccctgtctggcaggaataccgcaagaaggacaccactcgtctgaacctgatgttcttagggtcattcaaccttcagcctaccgtcaacaaaggcacgaagaaagagctggacaagcacaagcaggagtcaggcattagcccgaacttcgtccactcacaagatggtagccacctccgcaagactgtagtccacacgcaccgcaaatatggcgtgatgtcattcgcagtgattcacgatagcttcgggaccatcccggctgacgctgagtatctgttccgtggagtccgtgagacgatggtcgagacctaccgcgacaacgatgtgctgcttgacttctacgagcagtttgaataccagcttcacgagagccagagagacaagttgcctgagcttccgaagaaaggtaaactgaatatcgaagacatcttgtcttcagactttgcattcgcttaacaacaggagaagtatatgtcaatgaaacttgtagcacacaacagggtattcaacgatgggtcgggacgttgccatgtagagctgacttataaggatttaatcattctccgagacagattacagtcgggtgtgactgggtggattcaacctaacgagtacaaccttatagcttcgattgatgaagttcttaacgcgtggatggaagacgagcgcattcagtatccgtcattccctctaattagataaggagagagttatgaaatttgcacacaagcatactggcgttaatggtgggactcaaatcgtgaccgtaacagaacacaacggcaagggtctggtgaagaccacggtcatccctaccgagatgtccaagcagcttaacatcccgttcaagactcttgtatatctggtcgagtccagccacgagaagtacctgaaggacgcagtgtccaagctggagcaggccaaatgacagacatacagttactggccttgtggctgggagcactcgcagtattcactttaatccaacgcagaagaggttaaccctaaactatcactataggattagactcaaggtcatgactcaaagtcgtggccttcatgattaaccctaaataaacactactggagatttaaccgtatgtatcagaacactatcaacttcgagcgcatccgtgaacgtcagcagactgaaggttacatccctaagggccgcaagctgaacaagactaaacgtggaggaggtatcaaaggtgctttccgtaacgctgaaggtaaagactctatggttaaccaagagaaatacttcgtaggagcataaccaaatgggcagactttatagtggcaacctcaacgatttcaaagcagcgtgtcacaggctttatcagttagacttcgctgtcatatctcaggagtttcaagactatacgtcacgccaagagtgtatgaaactcagggtggaggaccgagctggtaacatcttcgcgcttgagaccttcgcacactacgatgaagacgtgctgtataataccgcaaccgactacctcaacggtctcgctgaccatctcgacacatggagcaaagaataatgacaactatcaaaactaaccctcaccgcgctgtagattactctgagtctggaattaagaaggcactggaagcagccgggtctctggaagctgaagtgaagtacgatggtgtgcgcctgaacctcctggtcctgcgtgaaggtgagacctactggcttagccgcgagtcgaaacctctaccagccttggagtggatgaactctgagttaggtaatgcgtggacccaagctgactggcgatggttcctgcgtcaatccggctacgaaggtgtgggcatgatgattgatggcgaggtcatggtcaaaggtgtagacttcaacacctcctcaggtctcatccgaacgaagtggctcaagcctaacaacgaggagttcgctgaatactattcgccggcgactggtggaaagaagctcccgttctggggatcccggtcacgacttcaggttgtggtctacggtgtcatcgacatgacaaccattgctgacccgaaagccgaaggtcctatccatagcgtcacacgcctgaaggccgaagctatcgtccctctcctccagaaatacttcccggaaatcgactgggttctgtctgagtcacacacggtctatgaccttgagtctctcaactccctgtacgaagagaagcgtctggaaggacacgagggtctggtagtcaaggacccacttggtaaatacaagcgcggcaagaagtcaggcatgtggaaaatgaagccggaggacaccattgatgggaccgtgtgtggactcgtgtgggggactcctggtaaggctaacgaaggtaagatcatcggctttgaggttctactggaggatggcatggtggtcaacgcctgcggtctgtctgaagaacagaaggacgggtttacggctaaggtcaaggaggacacgcttgctgcggttggcatctttgcgccgtacggcattggtggtaacgaaccttgcttcgataacccatacgaaggctggcagtgtgaagtcctcttcatggagaggttccctgatggctcccttcgtcaccccagcttcaagtgctggcgtggaaccgaagacaacccaacggtgaagtcatgagtacacaactttatatcaacatagcaagtagtcaactctacgctgtggtaaatggcgagctgtggtatcgtaaactcaagaagtgggccaagtcctcctacgatgaagagacaatatcaaccatgagtcatcgctaccgtaaggctgctaaggtgaacaactttaagatgcgttaacgtcaacccagtggtcttatgactgctgggtttctttgcgtacgggccaccagctagaccctaagctatcactataggacaaccctaaccgaccaaaggagaaaccttatgtctaaaaacttaatgttcaaccgatttactcgaagcttccacctgtcgcatagcccattcagcttccataaatctaatcaaccattaccccgctttggtaagacagtggctctgtctcccacagttcatgcgctagtcacccgcaagtctatgctgaaggctatggataaagaacaagtcgatgtacctgtggtcgttacaaaatggcctcgcattaagctggcccttctggtaattaaggaagtgttttgatggcatattgtgatagcaccacatactgtgaagcatgtaatggtgatgaccgcttcccacacgttggtaaacttgtaggtaacaagctgcaagaaattgatggtgtacgcaagccatcccactatcaggtctttgatggcgtggaatccattgagattatcgcacggtcaatgactgtgagtgagttccgtgggttctgcatgggtaacgtcctgaagtatcgactccgggctggtaagaagtcagagctggcaactatggagaaggacctgaacaaagcagccttctatcaggagctgttcgacctgcataaaggtaagtgctatgcttccgagtgagtggtgtgaaatgatgttcgagaagacaggtaacactgactaccttgaattgtataaccagtggaaggagcgcggtttatgactgaggttgagaagaaatacatcgtggagcttgagggtcgcgttcagtccttcgaggttccgttgtacgcaaagtctcttgaagaggctaccctgaagtcccaagagtatgaggacgctgggtttgtggtcggacggattcgccctgagacctaaactatcactgtaggacagacgtccagttagtaactttaaattaggagatttacaccaatggctaaagagcaactgaagactttcaccactccggtagctggtatcgttgagccttacgcatggctgaacaaagcagacaccaagtttaatgaacgtggtgagcataaggttaacctgacgttcgacctgagcgacccgaaggtccgtaagatgattgatgtcttacagaagattcacgacgatgcgtatgcgaaagcactcgcagaccacgagaagaacccacctcaggttcagcgtggcaagaagcctattgaaccacgtgaaggcgacatgccgtggattgagaatggtgacggtactgttacccttaagtttaaatgctttgcgtcttacctgaaagacggcaagtccgagcctatcttattacggttctacgacaccgatgctaaactcatccgtgacgtcccgaatattagcgctggctccaaactgaaggtcaagtttaaagtcctgccgttcaagtggaacgctgcgaccggtgcaagcgttaagctccagcttgagtcctgccttcttgtagaactgaaggagtggaaaggtgctggtggtgatggtggctggggtgatgatgaagaccttggtactggctacaaagcgccaaccgatggtgacttcgggtctgatgccttcggtgacgatggttccgaaggtggtgacgactccagctctggtggcgattacgacttctaatggcccaatggtctgcaaaacgggggcactctgtgggtgcctaccgctctggacttgaagccaagaaccagcagtggctggaacagaacggcgtcaaagcggagtacgaaagccattatatcaactatgtgattccggcttccgaccacaagtacacaccagattttatccttcctaacggtatcatcgtggagaccaaaggtatcttcgatagtgatgaccgtaagaagcaccttctggtacgagaacagcacccagagttagacatccggttcgtgttctcaagttcacgctccaagttatacaaagggtctccaaccacgtatggcgcatggtgcgaaaagaacggctataagtatgccgataaattcatcccggttgagtggcttcgagaggcgactgtacgtctgccttcaggtatactcatccccaagaagaaaggagttaagtgatgagcaagaagtttaaactgttagtagatgcgcatggctggcctagtgggactatagttaccaagtgtgagaatgaccccgtaccagattcaagaatgaccctagttgagtgccagattccaggcgcatacaaacatgggtctaacggctgcaatactcagcctgagggtatgtggggagcatgggtccttaattggaaacttgaggaaatcaagccggaagagaaactcactggtgtccaaaccactcaagtcctgccagcttcgagcgtaccgcctgtgactttgaagcgtgaagtcctgaccatcgacaagattggtgtaggccagacgttcatcgtccatggaaagcctgaagaagtttacgtgaagattagcaactcacacgtcttcaaccataagcatctccagatgcacaccacggacgcacaacgcttcacccagcacctgaatctggttgtcgtagaattggtggtgtacaatggtaagtaaggtacagttcaatccacggtcccggaccgacgctatcttcgtacactgttcggctaccaagccagagatggacatcggggtagagaccatccgtatgtggcacaagcagcaaggctggctggacgtaggctaccactttatcatcaagcgcgatggcactgtggaagagggacgcccggtcaatgtcgtagggtcacacgttaaggactggaactcacggtctgtaggcgtctgccttgtaggtggaattgacgctaagggcaagtttgaagctaacttcactccggcccagatgaactccctgcgcaacaagctggctgacctgaaggacttgtatcctcaggcagaaatcaaagcacatcatgacgtagcaccaaaggcgtgtccaagtttcgacttgcaacgctggctgtctaccaatgaactggtcacttccgaccgaggctaaactatcaccgtagggatgagaccacgagtcttgtccctttgttcgcatttgagattaagaaatgtctccatagctcaaacggtagagcggcgggtcgtgatggcctattgcgattagggttcgaatccccgtggagacgccactaaggagtgaccaatgtcatacgatgaccaagacgacgagagtgtctttctgtatcacacccagtgtccagactgtgggtcctcggatgccaatggtgtttactcagatgggcacatgtactgcttcgcctgtgacccttcagtcgcatggaagaaaggagacatggagttgaccgaggggtacacaccctcaggaggtagaaagcaagtgagcaatctgttaacgttcggtgagaacgctggacgatatgtcccactaccagcccgtagtctcagcatggagatatgcaagaagtacagctactgggtgggtaacatgggcggcaagatggttcaggtcgctgattattacgacaggtccgggaccaaggtagggcagaaagtccgagacgctgagaagaacttcacggctataggtagcgtcaagtctgacatgctgttcggctctcagctctggaacggtggtaagaagatagtcatcaccgagggtgagatagacgctctgtctgtggctcaggtgcaggacggtaagtatccagtggtatcacttccgttaggctccaagtctgcgaagaaagctatggctgcgaacattgagtatctcgaccagttcgaagagattatcctgatgttcgacatggacgaaccgggtcgtcaggccattgaggatgcagctccagtcttaccagcaggtagggtcaaggtagcgttcatcaatgggtacaaagacgccaacgctgcgcttcaggccaaggacttcaaggccatcaccgatgctatctggaacgctaaacctttcgtcccggctggagtggtatcagcggcaagcctgaaggaccgcacacgagaggcaatgcttaaagcagagactgaaggtctcatgttctcgtcatgcacaacactcaacgcgatgaccctcggtgcgcgagctggtgagcttatcatggttacttcagggtcaggcatgggtaagtccaccttcgtccgtcagctactcttagagtggggcagaggtggtaagcgtgtgggcatggctatgcttgaagaggctgtagaggaaacagttcaggaccttatgggtctggacaataacgtccgtctacgccagagcaaggaactgaagcaagccatcttagaggacggacggttcgacgaatggtatgacaagctgttcggagacgataagttccacctgtacgattcattcgcagagtcagaggaagacaccttgttcgctaagttatcctacatggtggatggtcttgactgtgacgtcatattgctggaccacatctcaatcgttgtgtcgggcatggaagataactcagatgaacgcaagaccattgaccgaatcatgactcgtctcaagaagtttgcgaagacgaagggcgtggttgtcgttgtcatatgtcacctgaagaacccagaaaaaggtaaatcgcatgaagaaggacgacctgtttcaatcactgacctacgtggttctggtgctctacgccaattatctgatactatcatcgcacttgagcgtaaccagcaaggtgatactcctaacgttgttcagcttcgtctactcaagtgtcgctttacaggtgatacgggagtggctggacacctcgagtacaacaagacgaccgggtggcttgaaccgattagcttcactggcagcagcggagaagaggatagcggctcgtgggaaaacaacgacttctagtcgggacatcgctgactataagaattttacggaggaccgttagtgttaaagaaacttaaagctcgctaccatcggttcatgtacaaatggtggagcgacgaagcaacctgcctgtcgaacattctgggagaccagcggttcaactctgaggcatggaagaaagctaaccggaagttcatgtatcacttcttgcgtacagacttctaggtctagactcaaggtcattcacatagagtggcctttatgattagactaaacggaggattaaccatgtttgaccttaagagtatctggggttctgacatcgagaccaacggtctccttgatacagtctcccagtttcactgtggggtcctgattaacgccgagtcgaatgagacccttaagtatggggtagctccgatggtcggtatcgtcggtggcttcaaagagtatgtgcagaaggtggaagagattgccgcatcacctgatggtatgctggtattccacaacggtatcaactatgacgtcccggctattgacaagctgaagcgtctgtacttcgggaaacgctttaacttcccgaaacacaagatgattgataccttggtgctgggtcgcttgatgtatcccaacattaagttctcagacatgggcgcagtgaaagctggtcgtctgccacctaagatgatgggacgccagtctcttgaggcttggggctatcgtctcggtgagatgaaaggtgagtacaaacacgattacgttgccaagtgcaaggctgaaggtatcgaatataaggctggggacgaatggttgttcccgtctcaggagatgctagactataacgttcaagacgttgtggtcacactggcgttgttcaagaagttcctgactgacaagtattacttccagtctgaacagttcgctttcgaccagatttatgcgttgcgtctggaacatgatgctgcgtggacctgtgcgaagatggaacgtaacggctatccgatgaacaccgagatggtcgaaggcttatatcgtgaactcaccgtcaaacgtgcagagctgctggacaagctgcgttcgactttcggtagctggtacgcaccaaagggcggaaaggagttcttcaagcacccacggacaggcaaggaccttccgaagtatccgagagtcgtgtatcctaaggtcggtggcatctttaagaagccgaagaacaaagctcaacgcttaggtcttgaaccctgtgaacgcgatacgcgagacacgatggagggagcaccattcacgccaatcacttacgttgagtttaatccgggaagcggagaccacttagcgaaagtcttgatggagcgtggctgggagcctgtggacttcactgacaccgggaaacctgtagtcgatgacgagacgttggaacacgttaagttaccagacgcagaggctcaggcttgcgtagagctggtccgtgagtatctggtagtccagaagcgcatcggtcaggcggctgaaggtaagaacgcatggttgaaacttgtaggtcaagacggacgtatgcacggttcaatcaacccatgcggggcagtaaccggacgtgcgacccatagtgcaccaaacatggctcaggtacctgctaacggtgctccgtatggtgagacttgccgtggtgctttcggtgcagcgtggaacaagaaggacggcaagccagacccttgggttcaagtaggcgtggatgcttcaggtcttgagcttcgttgtctggggaaccgagcggcaccgtttgatggtggcgactatgctaagactgtggtagaaggcgacatccactgggccaacgcagtcaacgctgggttagcacctaacgtcccacgcgacaagtcgagccatgaccacgatgctttccgtaataacgccaagacgttcatctatgcgttcctgtatggcgcaggggccgctaagattggactgatagttggtggtggtaagaaggaaggtgcggccctgatgaagaaattcattgagggtacaccagctatcaaggacctcagggaagctgtgagtaatacgttaatctcagactctaagtgggtggacggagagaacatcgttaagtggaaacgccgttggctgcgtggacttgatggtcgccgtatccacatccggtctccacactcagcactgaacgcattacttcaaggtgatggtgcggtagtctgtaagacttggttcacttggctggagcgtaacctcgaagctaagggctatgttcacgggtgggatggggactttgcgattatggcatttgtccacgatgaagttcaggttgctgcccgcaccatggagattgctgaggacatcgttaaggttgctcagtccacgatgcgcgaggtgggtgagttctatcagtttaaatgcgtattggacaccgagggcaagataggccctacgtggaaagaatgccactaaggaggtgcagatgggcggtgtagccactctccgcttccacaagatgcctacgggttgtatcgtttgtgtatcccaccgtagaaatcaggatgggtactttcggtatactgtaggctctgcccgtaagccgggacgtaaagcgtttatgtttcaccgctgggtctgggagcaacaggtcggaccgattcctgagggattcgagatagaccatttgtgtttaaaccgtgggtgctgtaacattgagcacttgcagtgtattgacgggaccgagcatactgtcaagaccaaccgtgagcggaagctcatcaagaagaaataaggagaaagctaatggctatgaccaaacgcgctatcgtaagtttcaaccttaaggctgtacttcctacagaccaagaggaaatcatcattggtggtctgcgtgagctggctaagagcgttaactcaggtgaaatcgagcctgacggtaagcagcgccatatgttgaccctgtggctaacagaaggtatggactcggtgattgagttcgttctgcgcgctagcttacggtcaatggttaaagatgctgtacaggaatattcagactcagagttcttcagtgtctcaccagccaccgtgaggttcaaacaatgagtgaatacttacgggtcctagcggccctcaagtcctgcccgaagaccttccagtccaactatgtgcgcaacaacgctgcacttgtggctgaggctgcgagtcgtggacatctaagctgcctgtctatggatgggcgtaacaacggtgcgtgggagattaccgctgctggcaccaagttcctgaaccaacacggaggatgcctgtgagcgaaaagaaaatagctctggtgctagacggtgactacttagtgttctcttctatggctgctgccgaggacgagacagactggggtgatggcatctggacccttatctgcgaccatgagaaggctcgtcgtatccttgagaacaccatcgctgaaatcgttaagaagcgtaaggcgtggaaagacgctaagattgtgatgtgctttactgacgataacaactggcgtaaggacgtgctacctacctataaggccaaccgtaaaggttctcgcaagcctgtaggttacaagaagttcgtagccgaagtgatggctgacccacggttcaacagcttcctacgtcctacacttgagggtgatgactgtatgggtatcatcgggacacgacctcagattgtaggctgtgaccatgctgttctggtgtcctgcgataaggacttcaagaccatcccgaactgtgagttcttctggttaaccactggtgaaattctaagtcatactactgctgaggcagactactggcacatggagcagaccatcaagggtgacactacagatggctacggtggcattccggggatgggcgaggatactactcgtgcgttccttgacgagccgtactacttcgtgcaggagagccgtgagcttaagactggcaagaacaaaggccagattaagactgagtggaagaagtatcctaagcgtgaagacatgacgctgtgggactgcatggtgactctggctgctaaagctgggatgaccgaggaggaacttctggtccaagctcaggtagctcgtatttgtcgagcctccgactacgaccctacgtccaaggaggtcatcctatggacaccatccatgtaatttactgggtcggacttctggccctttactgcatgtacaagtggttcgggtcgaacaaccgtcctaaacactgagtctaaccgatagtcatatcctatcaatccaatagtcatccataggtgaaacactaaactatcactatagggactttaggacctaagatatgactataagatagactttagtcttaacttaaagaggagattcaagatggcgattaatgctattgaaaacgttgttaagcagttacaggaagaaagacttgatgtcccgaacatctcccagtctgccatccagttcatgcacgtactgttcaacgcaagctacgctgagaagactggagctatcagtctcctcaagcagcaaggctacagcgatgcgttcattgccggattcatcaagggtctccagtattgttctgacactctcgactctgcgattgctatgcgtcgtgagctgaaagataccgttcagttcgattaactgtaggagggactatgtgtttcagtccaaagattagcactccgaagccttcggtccaagcgcctgaaccagcacctctgagtgaggaggttgcgtcagttgacatcggggctgaatcggatgtggacaccaacgagaccaaaggtatcaaagaccttaaggttaagaaggagtctgcacctaaagataaatcgtcagtgagtcgcgctatgcgagcctctggcgtaaacatggggtaagacaatgctaccatatctcaactcacgcgaaggtcgccacatgtgcgcctgccgcctctgggaagacgggcagtctaacttcaagtcattcgaggacttcaaggctcatacttaccgtattgctgacgagttcgacggtgaagagtacacaatctacgatgtctcaggtcaaccagtagcgtatctctacatgctggctaccacatcttggcaccgaccgactcccggtcttgacctttcaatcgtcgctattcgtcgtgactcgcagtcctcccgcaaggttcttgagactgtcaggtacatcatagacgaagagtgcaagcgttggggtcttggctggtattctcgtgtcaagcatgtttccgggtcggtagacatcgtaacaaccaagtgcgttagcgcgaacaaggagattaaccgtgggtaaatcaatcagtaaggccttcagtaaagtagtaaaaggtgctttagggaccgttggtcttggttctaacgatgcacctaaggttgttgaggctcagaccccagcagcaccagtggaagtaccgaacgacaaagtggaggatgtggatactgaaacaaccgcatctgacgagaagaaagtgaagcgctccggtaagcgtagccttcaggtctctcgtacatctggtggcggtatttctatataaggaggtgacgaatggctgaacgtgaagggttcgctgctgaaggcgctaagtcagtttatgatagattgaagaacggacgacagccttacgagacccgcgcacagaactgtgctgctgtcactatcccgtcactgtttcctaaggaatcagacaactcgtctactgaatataccactccgtggcaagctgtaggtgctcgctgcttgaacaacttggctgcaaagctgatgttggcgttattccctcagtcaccgtggatgcgactgacagtctccgaatatgaggccaagaccttgagtcaggactcagaggctgctgctcgtgttgacgaagggcttgctatggtcgagcgtgtgttgatggcctacatggagactaacagtttccgtgtgccattgttcgaagctctgaagcagcttatcgtctccggtaactgtctgctttacattccagagcctgaacagggtacttacagtccgatgcggatgtaccgcttagtgtcttacgttgttcaacgtgatgcgttcggtaacatcttgcagattgtgactctcgacaaggtagctttcagtgctctaccggaagacgtgaagtctcaactcaatgcagacgactatgagcctgacaccgagcttgaagtgtatacgcacatctaccgtcaagacgacgagtatctacgctacgaggaagtggaagggattgaggtagcagggaccgatggttcctacccgctgactgcatgtccgtacatcccggtacgaatggttcgactggatggtgaagactacggtcgttcttactgcgaggagtatctgggcgaccttaactcgctggagacgattacagaagctatcaccaaaatggctaaggtagcctccaaggtggtgggactcgttaacccgaacggtatcacgcaacctcgacgtctgaacaaggcggctacaggtgagttcgtggctggtcgcgttgaggacatcaacttcctgcaactgacgaaaggtcaggactttacgattgccaagtcggtggctgacgctatagagcaacgtttaggctgggccttccttcttaatagtgctgttcagcgtaatgccgagcgggtcactgctgaagagattcgttatgttgctggcgaactggaggcgaccttaggtggcgtgtactcagtacaatcacaagagcttcagttgcctatcgtccgtgtgctgatgaaccagcttcagtctgctggcatgattcctgaccttccgaaagaagcggtagagcctacggtctccactggtcttgaagcgttaggccgtggtcaagacttagagaagctgactcaggcagtcaacatgatgaccgggctacagcctctggctcaggacccagacattaacttgccgaccctgaagctgcgactgctgaatgccttaggcattgacaccgctggtctactccttacgcaggacgagaagattcagcgcatggctgaacagtcgtctcaacaggcagtagtccaaggtgctggtgctgctggtgccaacatgggcgctgctgtaggtcagggagctggtgaggacatggctcaagcctaaactatcactataggaacaacaccgtaagtccaactctaggtgagtcaactagacgaggcaggtgttacctattaactaccaaaggagagacttaatgtcccaatcagtttatgccgagttcggcgttagtcctaatgcaatcactggttccgttgaggacctgaacgaacaccagaagtctatgcttgaacaggacgtagctgttcgtgatggcgatgacgctattaccttcaagcaactggaagccgaaaacgaagaggctaccgaagaagacgagaacgtcgaagagactgaaggtgaagaagaccacgagtcagatgatgaagagtctgagaccgatggtgagcagccggagttcatcgaactaggtgatgcgccgaaagagctgactgaaagtgtcaccgctctggatgaaaacgaagctgcattcgacgacatggtgtcttctgctgtagaagctggcaaggtcactgctgatgaaattaccgctatcaaggctgaatacgccaaggacggtaagctgtctgacgcatcctacgctaagttgcaggaagcaggttacacaaagcgtttcgtagattcgtttgtccgtggtcaggaagctctggctgaacagtatgctgctggtgtggttcgctacgctggtggtgctgaacagtttaatcgcatcctgtcacaccttgagtccaacgacccgtcaactcgtgaagcattggaagctgccatcgttcgtaaggacattgcgactaccaaagctctgctgaatctggctggcaagactctgggtaaagctgtaggcgttaaacctcagcgtaccatcaccaatcaggctaaacctgtggttgcacctaaggctcctcagaccgaagcattcagctccaaggctgacatgattaaggctatgagtgacccgcgatacctgcgtgacgctaagtacacgatggaagttcgagctaaggtagctgcctcaagcctgtaggactaaactatcactatagggagaccaagagacagactcaaggtttcccctattacttaagtccatacggattgggcgtacagtaagtaataaactttatttttcaattgaataggagaattatcatatggcaaacgttccgggtcagaaagttggtacagaccaaggtaaaggcaactctggttccgacgctctggcgttgttcctgaaggtatttgctggcgaagtcctgaccgcattcactcgccgctctgtaactgctgacaagcatattgtccgtaccattcagaacggtaagtctgctcagttcccggtcatgggtcgcacctctggtgtgtatctggctccgggtgagagactgtccgataagcgtaaaggtatcaaacataccgagaaagtgattaccattgatggtctgctgactgccgatgtgatgattttcgacattgaagacgcgatgaaccactatgacgtggctggtgagtattccaaccagttgggtgaagctctggctatcgctgccgatggtgcggtactggctgagatggctattctgtgtaacctaccggctgcatctgatgaaaacatcgctggtcttggcaaagcgtctgtgctggaagttggtactaaagcagacctgaacactccggctaagctgggtgaagcaatcatcggtcaactgaccattgctcgtgcgaagctgacatccaactacgttcctgctggcgaccgttacttctacaccacgccggacaactactctgcaatcctcgcggctctgatgccgaacgctgctaactatgctgcgctgattgacccagagactggtaacatccgtaacgtaatgggcttcgtggttgttgaagttccacacttgactcagggtggtgctggggaaactcgtggtgccgatggtatcactattgcgactggtcagaagcacgccttcccagctactgctactggtgatgttaaagttgctctggacaacgttgtgggcctgttctctcaccgttctgctgtaggtactgttaagctgcgtgacttggcgctggaacgtgaccgtgacgtcgatgctcagggcgacctgattgttggtaagtacgctatgggtcacggtggtctgcgtccagaagcagcaggcgcactggttttcacagcggcgtcagcgggttaacgacctttaaggccctctctacagagggtcctaccttagagacgtatagttctacggtgggaaccagcctgaaggttgacttccctgagctttcagatgtgaccgattggtcgctgcttgaggtgactacgcctgatggtgttagctactcccgtagaaccaacagtctctacttcaaggccacctctggcgtggaaggtctggtgattgttgggtatgacgggacgcctgtgcgttccttcaacgtatctttcacaaactaattgaaaccccttgggtgccttcgggtgcttgaggggtttttttgcttaaggagggactatggtccttatttacacagggttagcactattcgtcttattctgggcgtacctgctgtccagctcaccgtctagcgcctatgaccgttaaggagtaaacctatggctcaatacattccactgaatgctaacgatgacttagatgccatcaacgatatgttagcagctatcggtgaaccagcagtcctacagcttgacgaaggtaacgctgacgtctcgaacgctcaacgtatcctgcatcgtgtcaatcgtcaggtccaagctaaaggctggaactttaacatcaacgaagctgctgtcctgacgcctgatgtccaagacaacaggattagattcctgccgtcttaccttcgggtcatgactgctggtgctaccagttactacagcaacatggggggctatctctatgacctgtccactcagtccacgaccttcactggaccaattacagtcgaactggtggagatgaaaccgttcgctgagatgcctgtagtattccgtgactacatcgttaccaaggctagccgtgagttcaacgctaagttcttcggtagcccagagtctgaactgtaccttcgtgagcaggaagcagaactctatcagcaggttatggaatacgagatggacactggtcgctacaacatgatgtctgacattgggagggactaatggctagtcacaacctgaagattcaccgccagcactttggtccggtacagctaggtctaaagacagcagagctgagacttaacgaccgggactttaaggttggcgactggcttatcctgaatgagtgggacaacgggtatactggacaacaggtagcacgtaaggttgtccacattgctgacgttggtgacatcgctgagggatacgtcctaatgagtatgatttaaggagggcatatgccgcttattacgcaaagcataaaaaatcttaagggtggcattagccaacagcctgacatcctgaggttctcagaccaaggcgaggctcaagttaactgctggtcatccgagagtgatggcctccagaagcgtccacctacagtcttcaagcgacgtcttaacatcgacgttgggagcaaccctaagttccacctgattaaccgtgatgagcaggagcagtattacatcgtgttcaacgggtccaacattcaggtagtcgacttgagcggtaatcaatactcagtttcaggtgcggtagactacgttaagtcgtccaacccgcgagatgacatccgtgtcgttacagttgcagactatacgttcatcgtgaaccgtaaggttgtcgttaacggtggaagcgagaagtcacactctggttataatcgtaaagctcgtgctttaattaacctgcgtggtggacagtatggtcgcacccttaaggtaggaatcaacggaggcgttaaggtttcgcataagttgccagcaggtaatgatgccgagaatgaccctcctaaggttgatgctcaggctatcggtgcagctctgagagaccttcttgttgctgcttaccctaccttcacgttcgaccttgggtctggattcctgttaatcactgccccttcagggactgacattaactcagtggagacggaggatggctacgctaaccagctaatcagcccagtactcgacacggtgcaaacaatctctaagctgcctcttgcagctccaaatgggtacatcattaagattcaaggtgagaccaacagtagcgccgatgagtattacgtgatgtatgactccaacactaagacgtggaaggagacagtagagccgggagtggtcactgggttcgataacaccacaatgccacatgctctggttagacaatctgacggctcctttgagttcaagactctggactggtctaagcggggtgctggtaatgatgacacaaaccctatgcctagcttcgtggatgctacgattaacgatgtgttcttctacaggaacaggctagggttcttgtcaggagagaacgtaatcatgagccgttcagccagctactttgcgttcttccctaagagtgtggcgacattgagtgatgatgaccctattgacgtagctgtaagtcaccctagaatctcaatacttaagtatgccgttccgtttagcgagcagctactactttggtcagatgaggtgcagttcgtgatgacaagctcgggggtccttacctcgaagtctatccagcttgatgtaggctcagagtttgccttaggagataacgccagaccgttcgctgtaggacgctcagtcttcttctcagcgcctcgtggatcattcaccagtattaagcgatacttcgctgtagcagatgtgtctgacgtgaaggatgccgatgataccactggtcacgtactgtcctatatccctaacggggtgtttgacattcaaggtacagggactgagaactacatctgcgtcaactccacaggtgcatacaaccgaatctacatctacaagttcttgtttaaggacggcgtacaacttcaagcctcttggtcgcactgggagttccctaaagctgataagattctggcgtctgcgtcgattggctctaccatgttcattgttcgtcagcaccaatggggtgtggacattgagcaccttaagttcatcaaggaggcaaccgactttccattagagccgtatagactccacgttgactctaaggtgtctatggtaatcccaattggctcatataacgctgacacctatgagactacggtcgacattggttctgcttatggtggaaacgctccgtctcccggtcggtactatctgattgacagtcagggtgcctatgtggaccttggtgaactgaccaacatctcaactgtggctatactcaatggcgattggtcgggacgtacagtgttcatcggacggtcttatctgatgtcctacaagttctcacggttcctgattaagattgaagacgatagtggcactcagtctgaagacactggacgtctacagcttcgtagggcttgggtcaactacaaggacactggcgctcttagactcattgtcagaaacggtgagcgggagttcgtgaacacctttaatgggtacacccttggtcagcaacccatcgggactaccaacattggggacggtcagtatcgcttcgctatgaatggtaacgcattaaccacgagtctaaccttagagtcagactatcctaccccagtgtccatcgttgggtgtggctgggaggcgtcatacgctaagaaagctcgttccgtctaacttattgaagggcctatagatttaccttaactatcactatagggactataggcccttaaggttataaggagactttatgtatattcgcaaggctacggaacaggatgtccactactttctgtggcatctttcagcagatgatgttaatgagtgcaaagcaaactacgggtcaaccgtgggtctctcagagagactgcttaagcatctatctccgtcatctgtggttttaacgaacggtgtaggtgaagtgtttgcctatggtggaaaccaaggggataacgtatggttcttgacttcgggtctggtccacaagctgagacctaaagagaagcgagagttcataaagcgtatctctgagtacagggacttaatgttagaccaatacgggaccatctggaactacgtgtggtcaggcaataagtctcacattaaattcttgaagttgcttggggctaagttccatgatgattggactatcagcccggtaactggtgagcattttcaattattcactatctctaaggaggacgtatgtgtgaacccgtaagtatcggcatgggtatcatggctgtagccggggccactatgtccgcatcccagcaggcaaaggccgaaggtgcagcaattgacgctcagaaccgacaggctcaggaaatggttaagcagatgaactactctgacgccaacctgagaatgcaggagcgagacctgaaggagcagcagatggctgaattgacagagaccacgctcaacggtatacgcaatcagggcatggtcagagctgcagtggctgagtcaggtctggaaggtaactctatggacaggattgaacgtcaggtcaaaggagatacagtcaaggagcgagcagggattaccgaaagttacaaccgagactatgcggctatcttcgggaaccgtatcgccaacattgagaacacaaagtctgctatccgtggtcaaggtaaaatcatcaagaccagcccactggcccatgcacttaatgttgctagcgccgggatgcaaggttacgccgctggtaagtcaatctctggagcgtccagctctggcggtgctgcacctattagtgctgctaaaggcacacctacaggtcatagctaagaggaggaataatggctagtaatattgaatcagctctggctaatcggactatgggtcgtggcagggctccgggtaaaactatcgccgtcaactatcaagcagccagcgttcaggctcctactggtgactccggtctggctcgtgcgttaaccaacttcgttgagtctgggacaggattgtacaagcagttcaaggacgaggagaagacacgggccgacgagcggtctaacgagattatccgtaaactgacacctcagcaaagacgtgaggctatccagaacggtacattgctgtatcaggatgacccttacgctatggaagcacttcgagtcaagacgggccgtaacgctgcctttgcggttgatgacgagattaacgttaagattcagaacggtgagttccgtacacgtcaggacatggaagagtatcgccaccagagacttcaggacgccgctaagtcctatgctgaagaggctggtattaaccctaccgacgagttcttccagcgcgggttcaacgataacatcacagaccgaaacatcgctatctatgggtctttcaataagtatttcagcaagcagtctgaagagacagcaatgttgaacactcgtattgagatgaactcgttccttaacgatggggacctgatgcgttcgcctgagtctggaaagaccttcatggcctaccttcgggatggactgacgactgctgctatcccttcggaccagcgagcacgagaggtaatcacccagactgtccgtgacgcaatccagaagtcaggaggctcaaacttcctacagcaagtccgtggcgagcgtatcacccttaacggtgtggacgctacagtcgaagagattgtaggccctgacgtcttcaatgctgctgtggttgaggctcaaggtaccgagtacaagttggtggctaagtatcaggaagacttatcgttaggcgttcagtctgcgattcttcaggacgacccaaccatcggtctggaccagattcagaaactcaaggagcagaacaacctgcttcagccgggtgaagaactcacgcctcagcgtcagatgcttattaatgccgaagccagcttactggaagcggtcaagcgtaagtccgctgaacaggcgaaggagaacactaagttaatccagacccagaacaagcaactagtcatagaccaagtgtatcagcgacgtctggctggggacaacgtgtccaccaactatgaggaccttccggtctcagatgctacaggagagttcaaacgttcagacatgaacaactatgcgtctgccaagctacagcagattgaccagatggacatccctgaggctgctaaggacgcccagaaggtggcattgttaagggctgacactaacaacggtccgttccgtaatgccttccagacgcttactcaggacgctgctggtgagtggcaagctgcggtcatccgtggacagtacgacccagacaagatgaaacgcttcgagtctcttcgtcgtgcctacactcaggacccttcaagtttcgctgctctgtatcctgaccaagctcagttgttctctacgttcgaccagatggacaagatgggtctggaccctcagacgatgattgaagctgataagcaagctgcaagtcaaagccgtgagatgcgcatggagtcagacaaggcgtggcaggagttgaagaacgactctcggaataaggacctttcgcgtcttcctacgtctctggacgcaagtgctcgtaaggtctgggactcatggtactatcgtacaggtaacgctgacgctgcaactcagcagactcaacgctggctgaatgagaacaccgtaacgttccagtctgatggttctgatggtaagtccatcggcatggtgtccaagcaccagcttatggtcggggataacccagagtcgtggcaggtgggtcgagacattatcgacaccgctcgtaagcagctcattaaggacaacccttgggtagtgaactctcagttgtccgttgttgaacagaacggctctatcttcctccaagacgctacggggactattcgtattcgatacgataaagaacttgtaggtaaactctaccgcgaacaacagcagaaggtacaagatgccgcatatgctcaggcagaacgtgacgctaacaagcgagcgcgtatcgtcgggactaaagctgctggtgacaaacgtcgagctgaccgagaggccaacatcgagaagagcggtgggatgtacaatgacgtctcactggagggtatcgcaaacgtactaattggtaaggagtaacataatggcgactcgtggtattcgcaataacaatccgggtaacatccgggtaagtaaggaccaatgggaagggatgactggagatgatggcgcattcgtcaccttcgatagtccagagtctggcgtccgagctttaggtaaaaacctgctgtcctacggtcgccaaggttatgactccatcgagaagattatcaaccgatgggcacctcctaacgagaacgacactaaggcttatattgactcagtggtggctgcaactggtattccagctacccagagtctagacctatctgaccctgacaccctgtcttctctggcacaagctatcagcttccatgagacaggatcacggtacgaccctgaagtctatcagaagggagtcgcacgggcactcaatggcattagcccaaagactccaccagtaagcgctaacgtatttgacgcactcacggaaggactcaaggctaaacctaaagtagatctgggcgagaaccttccgaccgctgctggtctaaacattgagggtcaagcacctgaagctcccaacgaatcgttcggtgagatgttctataagtctactggcgagaccatgcaggaacgagaggatcgctctacgtggttcggtttcggctcggctacagaagctgaagtgaagaactctatggtcggcgtggctatccgcgctggtcagaccgaggactcacttgatgtcattggcgatgtgtttaacccgacccgctggaacaaccataagtggtctcgtgaggagctggaccagattcgtaacgctggagttcttcctcagtattacggggtcattactggtggctcccctcagaacctgaccgagcttattaacttggcgcttgagaatcagaagttggaccaagagaaggccaaggctgggattggtgctcagttagctgctggtgtgattggggctggcgtggaccctctgacctacgttcctattgctgggcaggtaggcaaaggtgggaagctagtcaacaagatgttcactgtggcagctcagtctggtgctctggctggtgtgtctgagatggcccgtacctcagtggctggtggtgatgctcatgtggctgaagctatccttggcggtgctctcttcggtggtggcatgactgctatcgctgatgggttaggcagagccttaggccgcaacactaatgagtttgctggcccagctacacgtctggaagctcgtgagaccgctcgtaacgttgatggtcaggacctgtctcgtcttcctattcaggaaggtgagcagacctttagtcatcaaggtgttaagttcgcagacgttccgaacgagccgggtagtgtacgactggaagatggttcaatcctgattggtgagaatcctctgaaccctcagacacgtaaagtctttgacgaagtgattgagcctgaacgtgccgctgctggtgtgaaccttggtgggctgactgagattggcctgaagctgcttcggtccgagaaccctgagattcgtggagtagctgctgacttagtacgttcaccgactggtatgcagtctggggcctcaggtaaaatagggacaactgcgtcagacgtattcgagagacttcgtgctgtggaccatcggttctacaatgacatcgacgatgcggttactgaggcactaaaggacccgtacttccagacagcattctggcgagactctggcgcattccgtcaagacatctatcagcgcgtgtctatggctatcgaagatggtagcggaaacctgaaggctgaattgactccgggagaactgaaagtctatgacctgctgaagaaccagtttgacgccaagcgtgagatgatggagaaccccgctatgtttggtcgcccagacgctcagtctatctttccgggtagccgcttcaagggaacatacgtcccgcatgtgtatagcaaccagatgaaggagctgtacatcaaggagcttgggagtccagaggcactacaggaggccatcaagaagtcatggttgaccagctatgcgtctcgacctgaagtcaagaaacgtgtggacgaggcactcttagaggctgaccctacgttgactccagaaggacttgcggctgcggtcgataagtacgccaacgataaggcttatggtatctctcacaccgagcagttcgagcgttcatccgtaatggaagagaacatcaatggtctggtgggtctggagaacaacagcttccttgaggctcgtaacctgttcgatagcgatatgtcaatcgtcctacctaacggtcagaccttcagtgtcaacaacctgcgtgagtgggacatggacaagattgtcccggcctacaaccgtcgagttaatggcgatattgctatcatggctggtacaggcaagaccacgaaggacatgaaggacttggttgagaccctgatgaacaaggctggggatgacggtaagttgaaaggtgaagtatctaccttacgtgacactttgaagattctaactggtcgtgctcgacgtgatggtgctgatgatgcggccttcgctaccgtgatgcgcacaatgacagacctatcgttcttcgctaagaatgcctacatgggtgttcagaacttaacggagattggtggtatgctggctcgtggtaacgttcgtgcaatgcttcatggagtcccaattttccgtgacctagccttccgtaacaagaaggttggggcctcagagattaaggacctgcacaatgttatcttcggtaaggaactggatgactcaatccgtccgtctaaacaggatgtcattgaccgtctgcgatcttacagtgacctcggtcgtggtacagctacagctctggggactgccaagtattacactggcgaacttgcagtacgctctccgttcactaaagtcctcaacggtacgaccaactacctgttagatgctggacgtcagggcttcctgtctgacatcgtggagcatagcctgactggtagtaagcgtaagttcgatgaccgctggctgaagaccgctggtatctctgacgagcagtggaagggcattaagtccctaatccgtgagtcagtgactcgtggtccagacgggaagtacaccatcaaggataagaaggcgttcagtcaggacccaagggctatggacctctggcgtatgggtgacaccatcgctgacgagacgttactccggcctcataagctgtcaaacatggacgccaaggcttatggtcctctcgctaagactgtccttcagtttaagaacttcgtcatcaagtctatcaatgggagaaccatgcgaaccttctataacgccacgaagaacaacagagcgattgacgctgcactgtcgaccgtgatgtctatgggtctggctggtatctactacatggctcaggcgcatgtcaaggcttatgctatgcaggatggtcgagaccgtgactaccttaagcaagctctggacccaacgatgattggctatgcggccctgtcccgtagttcacatcttggtggcccacttggggtagctaacattctgggtggaatcgctgggtatgaggacactaagatgctccgctcgtcaatccttccgcgctcacctaccgagaagacggagaagccaatcgcctttggtgctgcttccagtggtccggtaatgaatgtggtcggcaacttccttgagcaggtcccggctttcggctatgctgctaacgttggtgctacggcttacaacttggcgggatacctcaaggctgatacccgtgtcaacgagcgagactacatgaccgggatgtataacacgttccgtgaacttgtaccgaatgacccgattacccagaagttgctgcttggaacgtttgaggagcagggcatccacatcaaggactaaactatcactataggaaactggaggcgctaccataggtctccgtttaaatcacaaaggaggcataatgtccacgattacacaattcccttcaggaaacactcagtacaggatagagttcgactacctagccagaacgtttgttgttgttacgctggtgaatagctctaaccctaccctgaaccgtgtactggaagttggtcgagattaccgattccttaatccaacgatgattgagatgttggctgaccaatcaggtttcgacatcgttcgtattcaccgtcagactggaactgacttagtggtagacttcaggaatggctcagtgttgacagctagtgacctgaccaattcagagcttcaggctatccatattgcagaagaaggtcgagaccaaacggttgacttagcgaaggaatatgccgatgctgctggtagctctgctggcaacgctaaggatagcgaggacgaatcacgccgaatcgctgcgagtatcaaggcagctggtaaaattggctatattacccgtcgctccttcgagaaaggcttcaacgttacaacatggaacgaggtcctgctatgggaagaggatggtgattattaccgctgggatggtacgcttccaaagaacgttcccgctggttcaactcctgaatcatctggtggtattgggctgagtgcgtgggttagtgttggtgatgcgtcacttagagcaaacctggctgatagtgatggcgctaaatacataggcagtggagaaaggacattacttgagcacaacaatgatgttttgcactcaaaagactttccaacactgcaggcagctatagatgcatctttgcaaaaaaatgatctactggtgtctcctggcaattatactgaaaaagttactattggaaacgcgcagttaaaaggtgttggcggggccacggtactaaaaactccggcagactttacaaacactgttcaggttaatttagctacacctcattggcaattccgccatagtggtggttttgctatagatggttccgggacaaccggggccgtaggtattagttttgacccgtcagaccaatattccggacgtcataattttagtgatgtatacatccacaacatcaacaaggccattcagaagccttccgggaacatcggcaatacttggagaaatattgggatatctacgtgtgattgggggtattacgcgattagtggctcagagatgcattgcggggccgataccctctacaatatccacttcgatggcatctccacctatgcagtctatctagacggcactgtcgataatggcggggggggcgcatggtggcttaaagactccattattgaggcttccggaggtggcgggatatacttaaaaagtaaatcgggcgactgtcctacatctccatgcggggtatccaatatatggatggaagcgatcgcaacatcaccggctgttcaggtagacggcgtggcgcaaaaaccgcgagttctcaagttggtagacacagcgatattctttgctgagtattcttatctcaacaacatcgagctatccaactccaacttagtaacttatggttgccgttttgacaacgctgatggcaatcaggatattgtcgtggatgcacaaagtaccattgtagcccatgacgtgtatttaaacggcagttctggaaaggacgttattgtggagtccgtagcatcgcaatctgcaacgatagctgccacaaacttatctctgaggggcaacttaacaagagggagagtatttaatacgccgacagggaataaattaatggctatcacatttgactcaggtagccataatttttctggcagcggcaccgttaacggttcgactgtatctgacggacttcacgccgctacatgtaccgaattttcattccccggagccggtttatatgaaatggtagcgacaagaacaaccattacatccggtagatggtacgtgtggggagttaactcacgcctacaatctggctcggcggatattagtataacgtcaggtattaccatgggtagtgtttacacaaagccgggggagtggattagcactttcggtgtaggaaaggcatctaccactggcactgtagcgctatacgtttccacaggaggaggttcgggagctacggtcagattcagtgactttttcatcgctgagtttacgacgcaagctcaggctttagctttcgccaattcaaggatgtcgttatcataaaaacaacctcagccgaatcgggttatttatcatcagaacggtattgaatcatcgaaggttgtggaggtagaggctaactacacgttgaccaacgtatgataacaactttgggtcacggacgacccgctttaaactggaggttttatgattgagttagacttcaagaatgaggtcctcaaagcctcgcctatcgtcgggaccgctgcggctgatggtgccagtcggttcttctttgggctaacgctcaacgaatggttctacgtcgctgctatcgcgtacaccgtggtgcagattggcgtcctaatttacaagacgattaagagcggaggtaagacatgacgcagatggacttagagaagttcctgttaatgctggacacagaacgtgctagactaatgctgcaagacctgcgggatgacactaagcgttcacctcagctctacaacgccattgagaaactgcttgctcgacacaactttgtgttaagcaaggtgtctgtggacgagaagacgctggcggatatggaggccttgaacgaagagtacgataaggtgctttcagctactgaggataatgacaccgggtatggtgttcaataagtgttagactcaaggtcatcgtcaggtggcctttatggttaacactgactagtggaggcgactctacgttaaatctgataaaccgggagggcaactatgctcgaatttttaaagagagcggctccgtggttacttgcagcagtgatgtttgctggtggctaccacaccgctaacaataagtgggaggctaaggtcaatgcagaatacacctcgaatcttaaggcatcggaagatacaaggcttgctgtccaagctgaagtcaacaaagtgtccaaacggtttcaggacgaaatgtcctcgctggaaggcagcactgataggattattgctgaccttcagtctgacaataagcggttgcgcatccgagtcaaaccaacgagtggaaccacgcaaagtgacggtcgatgcttcattgatggttacgccgaacttgacgaacgagatgctaaacgtcttatcgccatcggagtgaaaggagacaagtggattaaggcccttcaagacactgtgagagccttacagcaagagaaggaggtgacgcattgagtaaagacttagtggcgcgtcaggcgctaatgactgcacgtatgaagtcagacttcgtgttcttcctgttcgtcctgtggaaagctctgtcgctcccagtcccgactcgctgtcagattgacatggcgaagaaactatcggctggggacaacaggcgcttcatcctacaggcgttccgtggtatagggaagtccttcattacgtgtgccttcgttgtctggaagctatggaacaacccagacttgaagttcatgattgtgtcggcctcaaaggagcgagccgatgctaactccatcttcatcaagcgaatcatcgacctcatgcctcagcttcaggaactcaaacctaagcagggacagcgagatgcggttattagcttcgacgtgggacctgccaagccagaccactcaccttcggttaagtccgttggtatcactggtcagttgactggtagtcgtgctgacatcctgattgccgatgacgtggaggttccgaacaactcagcgactcaggctgcacgagaccgtctatcagagcttgtgaaagagttcgacgctatcctgaagccgggaggtacgatcatctatctgggtactcctcagaacgagatgaccctgtaccgtgagctggaaggtcgtgggtacaccactactatctggcccgctcgttatccacgcgacaggaaggactggcagtcttacggcgaccgtctggctcctatgcttcaggaagagctggaagaggaccctgagtccttctactggcgtccgactgatgaagtacgcttcgatgatacggacctgaaggaacgtgagctgtcctacggtaaagctggcttcgctctacagttcatgcttaacccgaacctgagtgatgccgagaagtaccctcttaagctccgtgaccttatcgtagccgacttggacccagcgtccagcccaatggtctaccaatggttgccgaaccctcagaacaagcgtgaggacgttcctaacgttggactcatgggtgactcgtaccacacgtatcagactgtaggttctgccttcagctcatacacccagaagattctggtcattgaccctagtggtcgtggtaaggatgaaactggatatgcggtactgtaccagctcaacggctacatcttcgctatggaagttggtggcatgcgtggtggttatgaagactctacgctggaagccttggctaagattggtcgtaagtggagggtcaacgaatacgtcattgagggtaacttcggtgatggtatgtaccttgagttattcaagcctgtagctgcccgtatccatcctgctgctgtaactgaagtgaagagtaagggtcagaaagaactccgcatctgtgacgttctggagcctatcatggggtctcacagacttatcgttaacgctgccgctatcgtccaagactaccagtcagcctctgataaggatggtgttcgtaaccctatctactctctcttctaccagatgactcgtatctctcgtgaacgtggagcattggcacatgatgaccgacttgatgcgctggctatcggtgtacagttcttcgttgagtcgatggctaaggatgccaacaaaggcgaacgtgaagtcactgaggagtggctggaggaacagatggagaacccacggaaaggcttcgagtccatccacactgagttctgggacaatggggtccgggtaactcacgatacggacgacgagcttggactagggtcatacgttacgttccactagctgaatgaataactataggtgaaagctgcattaataagcagctagtaacctatagttactaccagtctaacatactgttttacaaggagtttggacttaactatcactatagggaagacccccggttacttatagtattactatagtgaatatacatatgcagactttatgcaagaccttaggaggcagactccgagttcttacctaaggcttgcaccgatggaaggagggtgatattaatcataatccctccaatacagatagtcaccgaccatagatacaggaggtatgtagcatatggcaaagaccaaagctgtacttaaagctctggcgaccaatcgagctacatacaggtttcttactgctgttctacttgctgctggcgttactgctggaagtcagtgggtcgggtgggtcgagactctcgtatgttctctggtctctcagtgtaattaacgcaatcatgataacaatcaacgaaaggaggtagggatggacgaggagtcttatgggtcgttctctgacgaagattatcagacggagtgggaatacgcgcattgaagacctaaggtcagttcatagctgacgctactctactgaccttagctactgtagtcaaggactttaggtaacaccttaagagaagctcacttagggtcatcctacttattggtctatcctagtgtcgcctgacctacggtccttgacctacagtggctgtggcctacagtagtgacgatgagttttggacaaaaagtttgagaccacatctcacac